European Patent Application EP 4 159 749 A2, published April 5, 2023. Title: A method for producing Fc-containing molecule with remodeled sugar chain. Applicant: DAIICHI SANKYO COMPANY, LIMITED. The sequence listing filed with the application follows.

SEQUENCE LISTING (19 sequences)

SEQ ID NO: 1 - protein, 28 aa, Homo sapiens
SLRRSSCFGGRMDRIGAQSGLGCNSFRY

SEQ ID NO: 2 - DNA, 1422 bp, Artificial Sequence
  Nucleotide encoding the heavy chain of anti-LPS mAb-A
  CDS (1)..(1422): Encoding polypeptides including a signal sequence (19 aa) followed by Heavy chain of mAb-A (20-474: 455 aa)
atgaaacacctgtggttcttcctcctgctggtggcagctcccagatgggtgctgagccaggtgcagctggtgcagtctggcgccgaagtgaagaaaccaggcgccagcgtgaaggtgtcctgcaaggccagcggctacacctttaccagctactggatcaactgggtgcgccaggcccctggacagggcctggaatggatgggcaacatctaccccggcagcagcagcatcaactacaacgagaagttcaagagccgcgtgaccatcaccgccgacaccagcacaagcaccgcctacatggaactgagcagcctgcggagcgaggacaccgccgtgtactactgcgcccggaccatctacaactacggcagctccggctacaattacgccatggactactggggccagggcaccctcgtgaccgtgagctcagcctccaccaagggcccaagcgtcttccccctggcaccctcctccaagagcacctctggcggcacagccgccctgggctgcctggtcaaggactacttccccgaacccgtgaccgtgagctggaactcaggcgccctgaccagcggcgtgcacaccttccccgctgtcctgcagtcctcaggactctactccctcagcagcgtggtgaccgtgccctccagcagcttgggcacccagacctacatctgcaacgtgaatcacaagcccagcaacaccaaggtggacaagagagttgagcccaaatcttgtgacaaaactcacacatgcccaccctgcccagcacctgaactcctggggggaccctcagtcttcctcttccccccaaaacccaaggacaccctcatgatctcccggacccctgaggtcacatgcgtggtggtggacgtgagccacgaagaccctgaggtcaagttcaactggtacgtggacggcgtggaggtgcataatgccaagacaaagccccgggaggagcagtacaacagcacgtaccgggtggtcagcgtcctcaccgtcctgcaccaggactggctgaatggcaaggagtacaagtgcaaggtctccaacaaagccctcccagcccccatcgagaaaaccatctccaaagccaaaggccagccccgggaaccacaggtgtacaccctgcccccatcccgggaggagatgaccaagaaccaggtcagcctgacctgcctggtcaaaggcttctatcccagcgacatcgccgtggagtgggagagcaatggccagcccgagaacaactacaagaccacccctcccgtgctggactccgacggctccttcttcctctacagcaagctcaccgtggacaagagcaggtggcagcagggcaacgtcttctcatgctccgtgatgcatgaggctctgcacaaccactacacccagaagagcctctccctgtctcccggcaaa

SEQ ID NO: 3 - protein, 474 aa, Artificial Sequence
  Synthetic Construct
MKHLWFFLLLVAAPRWVLSQVQLVQSGAEVKKPGASVKVSCKASGYTFTSYWINWVRQAPGQGLEWMGNIYPGSSSINYNEKFKSRVTITADTSTSTAYMELSSLRSEDTAVYYCARTIYNYGSSGYNYAMDYWGQGTLVTVSSASTKGPSVFPLAPSSKSTSGGTAALGCLVKDYFPEPVTVSWNSGALTSGVHTFPAVLQSSGLYSLSSVVTVPSSSLGTQTYICNVNHKPSNTKVDKRVEPKSCDKTHTCPPCPAPELLGGPSVFLFPPKPKDTLMISRTPEVTCVVVDVSHEDPEVKFNWYVDGVEVHNAKTKPREEQYNSTYRVVSVLTVLHQDWLNGKEYKCKVSNKALPAPIEKTISKAKGQPREPQVYTLPPSREEMTKNQVSLTCLVKGFYPSDIAVEWESNGQPENNYKTTPPVLDSDGSFFLYSKLTVDKSRWQQGNVFSCSVMHEALHNHYTQKSLSLSPGK

SEQ ID NO: 4 - DNA, 702 bp, Artificial Sequence
  Nucleotides encoding the light chain of anti-LPS mAb-A
  CDS (1)..(702): Encoding polypeptides including a signal sequence (20 aa) followed by light chain of mAb-A (21-234: 214 aa)
atggtgctgcagacccaggtgttcatctccctgctgctgtggatctccggcgcgtacggcgacatcgtgatgacccagagccctgacagcctggccgtgtctctgggagagagagccaccatcaactgcaaggccagcgagaacgtgggcaacagcgtgtcctggtatcagcagaagcccggccagccccccaagctgctgatctacggcgccagcaacagatacaccggcgtgcccgatagattcagcggcagcggctctggcaccgacttcaccctgacaatcagctccctgcaggccgaggacgtggccgtgtactactgtggccagagctacagctacccctacaccttcggccagggcaccaaggtggaaatcaagcgtacggtggccgccccctccgtgttcatcttccccccctccgacgagcagctgaagtccggcaccgcctccgtggtgtgcctgctgaataacttctaccccagagaggccaaggtgcagtggaaggtggacaacgccctgcagtccgggaactcccaggagagcgtgaccgagcaggacagcaaggacagcacctacagcctgagcagcaccctgaccctgagcaaagccgactacgagaagcacaaggtgtacgcctgcgaggtgacccaccagggcctgagctcccccgtcaccaagagcttcaacaggggggagtgt

SEQ ID NO: 5 - protein, 234 aa, Artificial Sequence
  Synthetic Construct
MVLQTQVFISLLLWISGAYGDIVMTQSPDSLAVSLGERATINCKASENVGNSVSWYQQKPGQPPKLLIYGASNRYTGVPDRFSGSGSGTDFTLTISSLQAEDVAVYYCGQSYSYPYTFGQGTKVEIKRTVAAPSVFIFPPSDEQLKSGTASVVCLLNNFYPREAKVQWKVDNALQSGNSQESVTEQDSKDSTYSLSSTLTLSKADYEKHKVYACEVTHQGLSSPVTKSFNRGEC

SEQ ID NO: 6 - DNA, 1097 bp, Artificial Sequence
  Nucleotide sequence encoding the heavy chain of CLCH-1
  CDS (26)..(1072): Encoding polypeptides including a signal sequence (19 aa) followed by CH-A (20-349: 330 aa)
ccagcctccggactctagagccaccatgaagcacctgtggttctttctgctgctggtggccgctcccagatgggtgctgagcgcctctacaaagggccccagcgtgttccctctggcccctagcagcaagagcacatctggcggaacagccgccctgggctgcctcgtgaaggactactttcccgagcccgtgaccgtgtcctggaactctggcgctctgacaagcggcgtgcacacctttccagccgtgctgcagagcagcggcctgtactctctgagcagcgtcgtgacagtgcccagcagctctctgggcacccagacctacatctgcaacgtgaaccacaagcccagcaacaccaaggtggacaagcgggtggaacccaagagctgcgacaagacccacacctgtcccccttgtcctgcccccgaactgctgggaggcccttccgtgttcctgttccccccaaagcccaaggacaccctgatgatcagccggacccccgaagtgacctgcgtggtggtggatgtgtcccacgaggaccctgaagtgaagttcaattggtacgtggacggcgtggaagtgcacaacgccaagaccaagcctagagaggaacagtacaacagcacctaccgggtggtgtccgtgctgacagtgctgcaccaggactggctgaacggcaaagagtacaagtgcaaggtgtccaacaaggccctgcctgcccccatcgagaaaaccatcagcaaggccaagggccagccccgcgaaccccaggtgtacacactgcccccaagccgggaagagatgaccaagaaccaggtgtccctgacctgtctcgtgaaaggcttctacccctccgatatcgccgtggaatgggagagcaacggccagcccgagaacaactacaagaccaccccccctgtgctggacagcgacggctcattcttcctgtacagcaagctgaccgtggacaagagccggtggcagcagggcaacgtgttcagctgcagcgtgatgcacgaggccctgcacaaccactacacccagaagtccctgagcctgagccccggcaaatgagtttaaacgggggaggctaact

SEQ ID NO: 7 - protein, 349 aa, Artificial Sequence
  Synthetic Construct
MKHLWFFLLLVAAPRWVLSASTKGPSVFPLAPSSKSTSGGTAALGCLVKDYFPEPVTVSWNSGALTSGVHTFPAVLQSSGLYSLSSVVTVPSSSLGTQTYICNVNHKPSNTKVDKRVEPKSCDKTHTCPPCPAPELLGGPSVFLFPPKPKDTLMISRTPEVTCVVVDVSHEDPEVKFNWYVDGVEVHNAKTKPREEQYNSTYRVVSVLTVLHQDWLNGKEYKCKVSNKALPAPIEKTISKAKGQPREPQVYTLPPSREEMTKNQVSLTCLVKGFYPSDIAVEWESNGQPENNYKTTPPVLDSDGSFFLYSKLTVDKSRWQQGNVFSCSVMHEALHNHYTQKSLSLSPGK

SEQ ID NO: 8 - DNA, 425 bp, Artificial Sequence
  Nucleotide sequence encoding the light chain of CLCH-A
  CDS (26)..(400): Encoding polypeptides including a signal sequence (20 aa) followed by CL-A (21-125: 105 aa)
ccagcctccggactctagagccaccatggtgctgcagacccaggtgttcatcagcctgctgctgtggatcagcggcgcctatggcgtggcagcccctagcgtgttcatcttcccacccagcgacgagcagctgaagtctggcacagccagcgtcgtgtgcctgctgaacaacttctacccccgcgaggccaaggtgcagtggaaggtggacaatgccctgcagagcggcaacagccaggaaagcgtgaccgagcaggacagcaaggactccacctacagcctgagcagcaccctgaccctgagcaaggccgactacgagaagcacaaggtgtacgcctgcgaagtgacccaccagggcctgtctagccccgtgaccaagagcttcaaccggggcgagtgttgagtttaaacgggggaggctaact

SEQ ID NO: 9 - protein, 125 aa, Artificial Sequence
  Synthetic Construct
MVLQTQVFISLLLWISGAYGVAAPSVFIFPPSDEQLKSGTASVVCLLNNFYPREAKVQWKVDNALQSGNSQESVTEQDSKDSTYSLSSTLTLSKADYEKHKVYACEVTHQGLSSPVTKSFNRGEC

SEQ ID NO: 10 - DNA, 1047 bp, Artificial Sequence
  Nucleotide sequence encoding the heavy chain of CLCH-B (LALA form)
  CDS (1)..(1047): Encoding polypeptides including a signal sequence (19 aa) followed by CH-B (20-349: 330 aa)
atgaagcacctgtggttctttctgctgctggtggccgctcccagatgggtgctgagcgcctctacaaagggccccagcgtgttccctctggcccctagcagcaagagcacatctggcggaacagccgccctgggctgcctcgtgaaggactactttcccgagcccgtgaccgtgtcctggaactctggcgctctgacaagcggcgtgcacacctttccagccgtgctgcagagcagcggcctgtactctctgagcagcgtcgtgacagtgcccagcagctctctgggcacccagacctacatctgcaacgtgaaccacaagcccagcaacaccaaggtggacaagcgggtggaacccaagagctgcgacaagacccacacctgtcccccttgtcctgcccccgaagccgcgggaggcccttccgtgttcctgttccccccaaagcccaaggacaccctgatgatcagccggacccccgaagtgacctgcgtggtggtggatgtgtcccacgaggaccctgaagtgaagttcaattggtacgtggacggcgtggaagtgcacaacgccaagaccaagcctagagaggaacagtacaacagcacctaccgggtggtgtccgtgctgacagtgctgcaccaggactggctgaacggcaaagagtacaagtgcaaggtgtccaacaaggccctgcctgcccccatcgagaaaaccatcagcaaggccaagggccagccccgcgaaccccaggtgtacacactgcccccaagccgggaagagatgaccaagaaccaggtgtccctgacctgtctcgtgaaaggcttctacccctccgatatcgccgtggaatgggagagcaacggccagcccgagaacaactacaagaccaccccccctgtgctggacagcgacggctcattcttcctgtacagcaagctgaccgtggacaagagccggtggcagcagggcaacgtgttcagctgcagcgtgatgcacgaggccctgcacaaccactacacccagaagtccctgagcctgagccccggcaaa

SEQ ID NO: 11 - protein, 349 aa, Artificial Sequence
  Synthetic Construct
MKHLWFFLLLVAAPRWVLSASTKGPSVFPLAPSSKSTSGGTAALGCLVKDYFPEPVTVSWNSGALTSGVHTFPAVLQSSGLYSLSSVVTVPSSSLGTQTYICNVNHKPSNTKVDKRVEPKSCDKTHTCPPCPAPEAAGGPSVFLFPPKPKDTLMISRTPEVTCVVVDVSHEDPEVKFNWYVDGVEVHNAKTKPREEQYNSTYRVVSVLTVLHQDWLNGKEYKCKVSNKALPAPIEKTISKAKGQPREPQVYTLPPSREEMTKNQVSLTCLVKGFYPSDIAVEWESNGQPENNYKTTPPVLDSDGSFFLYSKLTVDKSRWQQGNVFSCSVMHEALHNHYTQKSLSLSPGK

SEQ ID NO: 12 - DNA, 30 bp, Artificial Sequence
  Forward primer of CHLALA-F
gcgggaggcccttccgtgttcctgttcccc

SEQ ID NO: 13 - DNA, 31 bp, Artificial Sequence
  Reverse primer of CHLALA-R
ggcttcgggggcaggacaagggggacaggtg

SEQ ID NO: 14 - DNA, 779 bp, Artificial Sequence
  Nucleotide sequence encoding Fc fragment (wild type)
  CDS (26)..(754): Encoding polypeptide containing a signal sequence (20 aa) followed by Fc-B (223 aa)
ccagcctccggactctagagccaccatggtgctgcagacccaggtgttcatcagcctgctgctgtggatcagcggcgcctacggcacctgtcctccatgtcctgctccagagctgctgggcggacctagcgtgttcctgttccccccaaagcccaaggacaccctgatgatcagccggacccccgaagtgacctgcgtggtggtggatgtgtcccacgaggaccctgaagtgaagttcaattggtacgtggacggcgtggaagtgcacaacgccaagaccaagcccagagaggaacagtacaacagcacctaccgggtggtgtccgtgctgaccgtgctgcaccaggactggctgaacggcaaagagtacaagtgcaaggtgtccaacaaggccctgcctgcccccatcgagaaaaccatcagcaaggccaagggccagccccgcgaaccccaggtgtacacactgccccctagcagggacgagctgaccaagaaccaggtgtccctgacctgtctcgtgaagggcttctacccctccgatatcgccgtggaatgggagagcaacggccagcccgagaacaactacaagaccaccccccctgtgctggacagcgacggctcattcttcctgtacagcaagctgacagtggacaagagccggtggcagcagggcaacgtgttcagctgcagcgtgatgcacgaggccctgcacaaccactacacccagaagtccctgagcctgagccccggcaaatgagtttaaacgggggaggctaact

SEQ ID NO: 15 - protein, 243 aa, Artificial Sequence
  Synthetic Construct
MVLQTQVFISLLLWISGAYGTCPPCPAPELLGGPSVFLFPPKPKDTLMISRTPEVTCVVVDVSHEDPEVKFNWYVDGVEVHNAKTKPREEQYNSTYRVVSVLTVLHQDWLNGKEYKCKVSNKALPAPIEKTISKAKGQPREPQVYTLPPSRDELTKNQVSLTCLVKGFYPSDIAVEWESNGQPENNYKTTPPVLDSDGSFFLYSKLTVDKSRWQQGNVFSCSVMHEALHNHYTQKSLSLSPGK

SEQ ID NO: 16 - DNA, 741 bp, Artificial Sequence
  Nucleotide sequence encoding Fc-A (LALA form)
  CDS (1)..(741): Encoding a signal peptide (20 aa) and Fc-A (227 aa)
atggtgctgcagacccaggtgttcatcagcctgctgctgtggatcagcggcgcctacggcgacaaaactcacacctgtcctccatgtcctgctccagaggccgcgggcggacctagcgtgttcctgttccccccaaagcccaaggacaccctgatgatcagccggacccccgaagtgacctgcgtggtggtggatgtgtcccacgaggaccctgaagtgaagttcaattggtacgtggacggcgtggaagtgcacaacgccaagaccaagcccagagaggaacagtacaacagcacctaccgggtggtgtccgtgctgaccgtgctgcaccaggactggctgaacggcaaagagtacaagtgcaaggtgtccaacaaggccctgcctgcccccatcgagaaaaccatcagcaaggccaagggccagccccgcgaaccccaggtgtacacactgccccctagcagggacgagctgaccaagaaccaggtgtccctgacctgtctcgtgaagggcttctacccctccgatatcgccgtggaatgggagagcaacggccagcccgagaacaactacaagaccaccccccctgtgctggacagcgacggctcattcttcctgtacagcaagctgacagtggacaagagccggtggcagcagggcaacgtgttcagctgcagcgtgatgcacgaggccctgcacaaccactacacccagaagtccctgagcctgagccccggcaaa

SEQ ID NO: 17 - protein, 247 aa, Artificial Sequence
  Synthetic Construct
MVLQTQVFISLLLWISGAYGDKTHTCPPCPAPEAAGGPSVFLFPPKPKDTLMISRTPEVTCVVVDVSHEDPEVKFNWYVDGVEVHNAKTKPREEQYNSTYRVVSVLTVLHQDWLNGKEYKCKVSNKALPAPIEKTISKAKGQPREPQVYTLPPSRDELTKNQVSLTCLVKGFYPSDIAVEWESNGQPENNYKTTPPVLDSDGSFFLYSKLTVDKSRWQQGNVFSCSVMHEALHNHYTQKSLSLSPGK

SEQ ID NO: 18 - DNA, 48 bp, Artificial Sequence
  Forward primer of FcLALA-F
tgtcctgctccagaggccgcgggcggacctagcgtgttcctgttcccc

SEQ ID NO: 19 - DNA, 51 bp, Artificial Sequence
  Reverse primer of Fc05-R
tggaggacaggtgtgagttttgtcgccgtaggcgccgctgatccacagcag